European Patent Application EP 4 219 757 A1, published August 2, 2023. Title: Multiplex nucleic acid detection method, composition and kit. Applicant: MACCURA BIOTECHNOLOGY CO., LTD. The sequence listing filed with the application follows.

SEQUENCE LISTING (36 sequences)

SEQ ID NO: 1 - DNA, 19 bp, Artificial Sequence
  Artificial sequence
acggatcacagcgtaaagc

SEQ ID NO: 2 - DNA, 20 bp, Artificial Sequence
  Artificial sequence
acggatcacacacgatgaca

SEQ ID NO: 3 - DNA, 20 bp, Artificial Sequence
  Artificial sequence
ccgtctcgcattaacatatt

SEQ ID NO: 4 - DNA, 40 bp, Artificial Sequence
  Artificial sequence
acggatcacagcgtaaagctgcaacatgaccaaggactgg

SEQ ID NO: 5 - DNA, 19 bp, Artificial Sequence
  Artificial sequence
atgtagaagccctggtagc

SEQ ID NO: 6 - DNA, 39 bp, Artificial Sequence
  Artificial sequence
acggatcacagcgtaaagcctaagcagactcacagaact

SEQ ID NO: 7 - DNA, 20 bp, Artificial Sequence
  Artificial sequence
atgagaacttgccataggtt

SEQ ID NO: 8 - DNA, 39 bp, Artificial Sequence
  Artificial sequence
acggatcacacacgatgacataactcaaggcggacgatt

SEQ ID NO: 9 - DNA, 18 bp, Artificial Sequence
  Artificial sequence
ttaaccacggcgttcagg

SEQ ID NO: 10 - DNA, 38 bp, Artificial Sequence
  Artificial sequence
acggatcacacacgatgacatggacaacagcagacaac

SEQ ID NO: 11 - DNA, 20 bp, Artificial Sequence
  Artificial sequence
tccacacgtacaaggtatct

SEQ ID NO: 12 - DNA, 40 bp, Artificial Sequence
  Artificial sequence
ccgtctcgcattaacatattataatcaggcacgagaacag

SEQ ID NO: 13 - DNA, 19 bp, Artificial Sequence
  Artificial sequence
gactagcaacctccatggc

SEQ ID NO: 14 - DNA, 42 bp, Artificial Sequence
  Artificial sequence
ccgtctcgcattaacatattaagcaaccaacaacattcattg

SEQ ID NO: 15 - DNA, 19 bp, Artificial Sequence
  Artificial sequence
gcaattcagcatcacagac

SEQ ID NO: 16 - DNA, 41 bp, Artificial Sequence
  Artificial sequence
ctccaccacttactgattatctcaaagccgagatcgcacag

SEQ ID NO: 17 - DNA, 23 bp, Artificial Sequence
  Artificial sequence
tccccttagtcagaggtgacagg

SEQ ID NO: 18 - DNA, 42 bp, Artificial Sequence
  Artificial sequence
ctccacgacttacagattacttgaagggtttgagccatactg

SEQ ID NO: 19 - DNA, 21 bp, Artificial Sequence
  Artificial sequence
ccctggggttgaagggtaatc

SEQ ID NO: 20 - DNA, 45 bp, Artificial Sequence
  Artificial sequence
acgacctatgaacgctctctcattaagcaagaaaaggaaaagaag

SEQ ID NO: 21 - DNA, 22 bp, Artificial Sequence
  Artificial sequence
tgcagatccaacacctaacaaa

SEQ ID NO: 22 - DNA, 45 bp, Artificial Sequence
  Artificial sequence
acgacctatgcacgcactctccaacctatgagcaggcaggtggtt

SEQ ID NO: 23 - DNA, 23 bp, Artificial Sequence
  Artificial sequence
tggtaaggtgacggctttgtagt

SEQ ID NO: 24 - DNA, 40 bp, Artificial Sequence
  Artificial sequence
caactaaccaggatcaacgagcaccccaacagtgaaacga

SEQ ID NO: 25 - DNA, 20 bp, Artificial Sequence
  Artificial sequence
ggcacgagtaaaacggcaaa

SEQ ID NO: 26 - DNA, 41 bp, Artificial Sequence
  Artificial sequence
caaccaaccagcatcaacatgaccgaaaggtaagatggaga

SEQ ID NO: 27 - DNA, 21 bp, Artificial Sequence
  Artificial sequence
acaggcaaactgagttggacg

SEQ ID NO: 28 - DNA, 18 bp, Artificial Sequence
  Artificial sequence
ctccaccacttactgatt

SEQ ID NO: 29 - DNA, 19 bp, Artificial Sequence
  Artificial sequence
acgacctatgaacgctctc

SEQ ID NO: 30 - DNA, 18 bp, Artificial Sequence
  Artificial sequence
caaccaaccagcatcaac

SEQ ID NO: 31 - DNA, 43 bp, Artificial Sequence
  Artificial sequence
caaccaaccagcatgaaccgcttgaatatgttgatatgctcca

SEQ ID NO: 32 - DNA, 23 bp, Artificial Sequence
  Artificial sequence
gcggataacggtatctgttgttt

SEQ ID NO: 33 - DNA, 21 bp, Artificial Sequence
  Artificial sequence
ggagcgagatccctccaaaat

SEQ ID NO: 34 - DNA, 23 bp, Artificial Sequence
  Artificial sequence
ggctgttgtcatacttctcatgg

SEQ ID NO: 35 - DNA, 21 bp, Artificial Sequence
  Artificial sequence
gcaggggggagccaaaagggt

SEQ ID NO: 36 - DNA, 40 bp, Artificial Sequence
  Artificial sequence
caactaaccagcatcaacgagcaccccaacagtgaaacga